European Patent Specification EP 3 596 213 B1, published August 12, 2026. Title: COMPOSITIONS AND METHODS FOR ENHANCED GENE EXPRESSION. Applicant: Keravala, Annahita. The sequence listing filed with the application follows.

SEQUENCE LISTING (97 sequences)

SEQ ID NO: 1 - DNA, 293 bp, Human cytomegalovirus
acttacggtaaatggcccgcctggctgaccgcccaacgacccccgcccattgacgtcaataatgacgtatgttcccatagtaacgccaatagggactttccattgacgtcaatgggtggagtatttacggtaaactgcccacttggcagtacatcaagtgtatcatatgccaagtccgccccctattgacgtcaatgacggtaaatggcccgcctggcattatgcccagtacatgaccttacgggactttcctacttggcagtacatctacgtattagtcatcgctattacca

SEQ ID NO: 2 - DNA, 659 bp, Human cytomegalovirus
tcaatattggccattagccatattattcattggttatatagcataaatcaatattggctattggccattgcatacgttgtatctatatcataatatgtacatttatattggctcatgtccaatatgaccgccatgttggcattgattattgactagttattaatagtaatcaattacggggtcattagttcatagcccatatatggagttccgcgttacataacttacggtaaatggcccgcctggctgaccgcccaacgacccccgcccattgacgtcaataatgacgtatgttcccatagtaacgccaatagggactttccattgacgtcaatgggtggagtatttacggtaaactgcccacttggcagtacatcaagtgtatcatatgccaagtccgccccctattgacgtcaatgacggtaaatggcccgcctggcattatgcccagtacatgaccttacgggactttcctacttggcagtacatctacgtattagtcatcgctattaccatggtgatgcggttttggcagtacaccaatgggcgtggatagcggtttgactcacggggatttccaagtctccaccccattgacgtcaatgggagtttgttttggcaccaaaatcaacgggactttccaaaatgtcgtaataacc

SEQ ID NO: 3 - DNA, 171 bp, Homo sapiens
gcacatcgcccacagtccccgagaagttggggggaggggtcggcaattgaaccggtgcctagagaaggtggcgcggggtaaactgggaaagtgatgtcgtgtactggctccgcctttttcccgagggtgggggagaaccgtatataagtgcagtagtcgccgtgaacgttc

SEQ ID NO: 4 - DNA, 220 bp, Human cytomegalovirus
tgctgatgcggttttggcagtacaccaatgggcgtggatagcggtttgactcacggggatttccaagtctccaccccattgacgtcaatgggagtttgttttggcaccaaaatcaacgggactttccaaaatgtcgtaataaccccgccccgttgacgcaaatgggcggtaggcgtgtacggtgggaggtctatataagcagagctcgtttagtgaaccg

SEQ ID NO: 5 - DNA, 923 bp, Homo sapiens
gtaagtgccgtgtgtggttcccgcgggcctggcctctttacgggttatggcccttgcgtgccttgaattacttccacctggctccagtacgtgattcttgatcccgagctggagccaggggcgggccttgcgctttaggagccccttcgcctcgtgcttgagttgaggcctggcctgggcgctggggccgccgcgtgcgaatctggtggcaccttcgcgcctgtctcgctgctttcgataagtctctagccatttaaaatttttgatgacgtgctgcgacgctttttttctggcaagatagtcttgtaaatgcgggccaggatctgcacactggtatttcggtttttgggcccgcggccggcgacggggcccgtgcgtcccagcgcacatgttcggcgaggcggggcctgcgagcgcggccaccgagaatcggacgggggtagtctcaagctggccggcctgctctggtgcctggcctcgcgccgccgtgtatcgccccgccctgggcggcaaggctggcccggtcggcaccagttgcgtgagcggaaagatggccgcttcccggccctgctccagggggctcaaaatggaggacgcggcgctcgggagagcgggcgggtgagtcacccacacaaaggaaaagggcctttccgtcctcagccgtcgcttcatgtgactccacggagtaccgggcgccgtccaggcacctcgattagttctggagcttttggagtacgtcgtctttaggttggggggaggggttttatgcgatggagtttccccacactgagtgggtggagactgaagttaggccagcttggcacttgatgtaattctccttggaatttggcctttttgagtttggatcttggttcattctcaagcctcagacagtggttcaaagtttttttcttccatttcag

SEQ ID NO: 6 - DNA, 27 bp, Homo sapiens
acacccaagctgtctagagccgccacc

SEQ ID NO: 7 - DNA, 300 bp, Homo sapiens
ggttcccttttattttttacatataaatatatttccctgtttttctaaaaaagaaaaagatcatcattttcccattgtaaaatgccatatttttttcataggtcacttacatatatcaatgggtctgtttctgagctctactctattttatcagcctcactgtctatccccacacatctcatgctttgctctaaatcttgatatttagtggaacattctttcccattttgttctacaagaatatttttgttattgtctttgggctttctatatacattttgaaatgaggttgacaagtta

SEQ ID NO: 8 - DNA, 589 bp, Woodchuck hepatitis virus
aatcaacctctggattacaaaatttgtgaaagattgactggtattcttaactatgttgctccttttacgctatgtggatacgctgctttaatgcctttgtatcatgctattgcttcccgtatggctttcattttctcctccttgtataaatcctggttgctgtctctttatgaggagttgtggcccgttgtcaggcaacgtggcgtggtgtgcactgtgtttgctgacgcaacccccactggttggggcattgccaccacctgtcagctcctttccgggactttcgctttccccctccctattgccacggcggaactcatcgccgcctgccttgcccgctgctggacaggggctcggctgttgggcactgacaattccgtggtgttgtcggggaaatcatcgtcctttccttggctgctcgcctgtgttgccacctggattctgcgcgggacgtccttctgctacgtcccttcggccctcaatccagcggaccttccttcccgcggcctgctgccggctctgcggcctcttccgcctcttcgccttcgccctcagacgagtcggatctccctttgggccgcctccccgc

SEQ ID NO: 9 - DNA, 251 bp, Bos taurus
ttgccagccatctgttgtttgcccctcccccgtgccttccttgaccctggaaggtgccactcccactgtcctttcctaataaaatgaggaaattgcatcgcattgtctgagtaggtgtcattctattctggggggtggggtggggcaggacagcaagggggaggattgggaatacaatagcaggcatgctggggatgcggtgggctctatgggtacccaggtgctgaagaattgacccggttcctcctggg

SEQ ID NO: 10 - DNA, 127 bp, Adeno-associated virus 2
gcgcgctcgctcgctcactgaggccgcccgggcaaagcccgggcgtcgggcgacctttggtcgcccggcctcagtgagcgagcgagcgcgcagagagggagtggccaactccatcactaggggttcc

SEQ ID NO: 11 - DNA, 318 bp, Human adenovirus 2
ctcactctcttccgcatcgctgtctgcgagggccagctgttgggctcgcggttgaggacaaactcttcgcggtctttccagtactcttggatcggaaacccgtcggcctccgaacggtactccgccaccgagggacctgagcgagtccgcatcgaccggatcggaaaacctctcgagaaaggcgtctaaccagtcacagtcgcaaggtaggctgagcaccgtggcgggcggcagcgggtggcggtcggggttgtttctggcggaggtgctgctgatgatgtaattaaagtaggcggtcttgagacggcggatggtcga

SEQ ID NO: 12 - DNA, 102 bp, Human adenovirus 2
ccagctgttggggtgagtactccctctcaaaagcgggcattacttctgcgctaagattgtcagtttccaaaaacgaggaggatttgatattcacctggcccg

SEQ ID NO: 13 - DNA, 810 bp, Homo sapiens
ctgttctcatcacatcatatcaaggttatataccatcaatattgccacagatgttacttagccttttaatatttctctaatttagtgtatatgcaatgatagttctctgatttctgagattgagtttctcatgtgtaatgattatttagagtttctctttcatctgttcaaatttttgtctagttttattttttactgatttgtaagacttctttttataatctgcatattacaattctctttactggggtgttgcaaatattttctgtcattctatggcctgacttttcttaatggttttttaattttaaaaataagtcttaatattcatgcaatctaattaacaatcttttctttgtggttaggactttgagtcataagaaatttttctctacactgaagtcatgatggcatgcttctatattattttctaaaagatttaaagttttgccttctccatttagacttataattcactggaatttttttgtgtgtatggtatgacatatgggttcccttttattttttacatataaatatatttccctgtttttctaaaaaagaaaaagatcatcattttcccattgtaaaatgccatatttttttcataggtcacttacatatatcaatgggtctgtttctgagctctactctattttatcagcctcactgtctatccccacacatctcatgctttgctctaaatcttgatatttagtggaacattctttcccattttgttctacaagaatatttttgttattgtctttgggctttctatatacattttgaaatgaggttgacaagtta

SEQ ID NO: 14 - DNA, 202 bp, Homo sapiens
ctgcccgggtggcatccctgtgacccctccccagtgcctctcctggccctggaagttgccactccagtgcccaccagccttgtcctaataaaattaagttgcatcattttgtctgactaggtgtccttctataatattatggggtggaggggggtggtatggagcaaggggcccaagttgggaagaaacctgtagggcctgc

SEQ ID NO: 15 - DNA, 145 bp, Adeno-associated virus 2
gttaatcattaactacaaggaacccctagtgatggagttggccactccctctctgcgcgctcgctcgctcactgaggccgggcgaccaaaggtcgcccgacgcccgggctttgcccgggcggcctcagtgagcgagcgagcgcgc

SEQ ID NO: 16 - DNA, 155 bp, Homo sapiens
ggcatgcttctatattattttctaaaagatttaaagttttgccttctccatttagacttataattcactggaatttttttgtgtgtatggtatgacatatgggttcccttttattttttacatataaatatatttccctgtttttctaaaaaaga

SEQ ID NO: 17 - DNA, 726 bp, Human hepatitis B virus
ataacaggcctattgattggaaagtttgtcaacgaattgtgggtcttttggggtttgctgccccttttacgcaatgtggatatcctgctttaatgcctttatatgcatgtatacaagcaaaacaggcttttactttctcgccaacttacaaggcctttctcagtaaacagtatatgaccctttaccccgttgctcggcaacggcctggtctgtgccaagtgtttgctgacgcaacccccactggttggggcttggccataggccatcagcgcatgcgtggaacctttgtgtctcctctgccgatccatactgcggaactcctagccgcttgttttgctcgcagcaggtctggagcaaacctcatcgggaccgacaattctgtcgtactctcccgcaagtatacatcgtttccatggctgctaggctgtgctgccaactggatcctgcgcgggacgtcctttgtttacgtcccgtcggcgctgaatcccgcggacgacccctcccggggccgcttggggctctaccgcccgcttctccgtctgccgtaccgtccgaccacggggcgcacctctctttacgcggactccccgtctgtgccttctcatctgccggaccgtgtgcacttcgcttcacctctgcacgtcgcatggaggccaccgtgaacgcccaccggaacctgcccaaggtcttgcataagaggactcttggactttcagcaatgtcatc

SEQ ID NO: 18 - DNA, 170 bp, Human cytomegalovirus
gtaagtctgttgacatgtatgtgatgtatactaacctgcatgggacgtggatttacttgtgtatgtcagatagagtaaagattaactcttgcatgtgagcggggcatcgagatagcgataaatgagtcaggaggacggatacttatatgtgttgttatcctcctctacag

SEQ ID NO: 19 - DNA, 50 bp, Homo sapiens
agcttgcttgttctttttgcagaagctcagaataaacgctcaactttggc

SEQ ID NO: 20 - DNA, 387 bp, Oryctolagus cuniculus
tggctaataaaggaaatttattttcattgcaatagtgtgttggaattttttgtgtctctcactcggaaggacatatgggagggcaaatcatttaaaacatcagaatgagtatttggtttagagtttggcaacatatgcccatatgctggctgccatgaacaaaggttggctataaagaggtcatcagtatatgaaacagccccctgctgtccattccttattccatagaaaagccttgacttgaggttagattttttttatattttgttttgtgttatttttttctttaacatccctaaaattttccttacatgttttactagccagatttttcctcctctcctgactactcccagtcatagctgtccctcttctcttatggagatc

SEQ ID NO: 21 - DNA, 83 bp, Human cytomegalovirus
ccgccccgttgacgcaaatgggcggtaggcgtgtacggtgggaggtctatataagcagagctcgtttagtgaaccgtcagatc

SEQ ID NO: 22 - DNA, 133 bp, Artificial Sequence
  Synthetic construct
gtaagtatcaaggttacaagacaggtttaaggagaccaatagaaactgggcttgtcgagacagagaagactcttgcgtttctgataggcacctattggtcttactgacatccactttgcctttctctccacag

SEQ ID NO: 23 - DNA, 197 bp, Human cytomegalovirus
ggggctcgggtgcagcggccagcgggcgcctggcggcgaggattacccggggaagtggttgtctcctggctggagccgcgagacgggcgctcagggcgcggggccggcggcggcgaacgagaggacggactctggcggccgggtctttggccgcggggagcgcgggcaccgggcgagcaggccgcgtcgcgctcacc

SEQ ID NO: 24 - DNA, 2064 bp, Homo sapiens
atggtcagctactgggacaccggggtcctgctgtgcgcgctgctcagctgtctgcttctcacaggatctagttcaggttcaaaattaaaagatcctgaactgagtttaaaaggcacccagcacatcatgcaagcaggccagacactgcatctccaatgcaggggggaagcagcccataaatggtctttgcctgaaatggtgagtaaggaaagcgaaaggctgagcataactaaatctgcctgtggaagaaatggcaaacaattctgcagtactttaaccttgaacacagctcaagcaaaccacactggcttctacagctgcaaatatctagctgtacctacttcaaagaagaaggaaacagaatctgcaatctatatatttattagtgatacaggtagacctttcgtagagatgtacagtgaaatccccgaaattatacacatgactgaaggaagggagctcgtcattccctgccgggttacgtcacctaacatcactgttactttaaaaaagtttccacttgacactttgatccctgatggaaaacgcataatctgggacagtagaaagggcttcatcatatcaaatgcaacgtacaaagaaatagggcttctgacctgtgaagcaacagtcaatgggcatttgtataagacaaactatctcacacatcgacaaaccaatacaatcatagatgtccaaataagcacaccacgcccagtcaaattacttagaggccatactcttgtcctcaattgtactgctaccactcccttgaacacgagagttcaaatgacctggagttaccctgatgaaaaaaataagagagcttccgtaaggcgacgaattgaccaaagcaattcccatgccaacatattctacagtgttcttactattgacaaaatgcagaacaaagacaaaggactttatacttgtcgtgtaaggagtggaccatcattcaaatctgttaacacctcagtgcatatatatgataaagcattcatcactgtgaaacatcgaaaacagcaggtgcttgaaaccgtagctggcaagcggtcttaccggctctctatgaaagtgaaggcatttccctcgccggaagttgtatggttaaaagatgggttacctgcgactgagaaatctgctcgctatttgactcgtggctactcgttaattatcaaggacgtaactgaagaggatgcagggaattatacaatcttgctgagcataaaacagtcaaatgtgtttaaaaacctcactgccactctaattgtcaatgtgaaaccccagatttacgaaaaggccgtgtcatcgtttccagacccggctctctacccactgggcagcagacaaatcctgacttgtaccgcatatggtatccctcaacctacaatcaagtggttctggcacccctgtaaccataatcattccgaagcaaggtgtgacttttgttccaataatgaagagtcctttatcctggatgctgacagcaacatgggaaacagaattgagagcatcactcagcgcatggcaataatagaaggaaagaataagatggctagcaccttggttgtggctgactctagaatttctggaatctacatttgcatagcttccaataaagttgggactgtgggaagaaacataagcttttatatcacagatgtgccaaatgggtttcatgttaacttggaaaaaatgccgacggaaggagaggacctgaaactgtcttgcacagttaacaagttcttatacagagacgttacttggattttactgcggacagttaataacagaacaatgcactacagtattagcaagcaaaaaatggccatcactaaggagcactccatcactcttaatcttaccatcatgaatgtttccctgcaagattcaggcacctatgcctgcagagccaggaatgtatacacaggggaagaaatcctccagaagaaagaaattacaatcagaggtgagcactgcaacaaaaaggctgttttctctcggatctccaaatttaaaagcacaaggaatgattgtaccacacaaagtaatgtaaaacattaa

SEQ ID NO: 25 - DNA, 20 bp, Human cytomegalovirus
aggactcattaaaaagtaac

SEQ ID NO: 26 - DNA, 222 bp, Simian virus 40
cagacatgataagatacattgatgagtttggacaaaccacaactagaatgcagtgaaaaaaatgctttatttgtgaaatttgtgatgctattgctttatttgtaaccattataagctgcaataaacaagttaacaacaacaattgcattcattttatgtttcaggttcagggggagatgtgggaggttttttaaagcaagtaaaacctctacaaatgtggta

SEQ ID NO: 27 - DNA, 1075 bp, Artificial Sequence
  Made in Lab - Polynucleotide cassette 1 full 5'
ctctggagacgcaacctttggagctaagccagcaatggtagagggaagattctgcacgtcccttccaggcggcctccccgtcaccaccccccccaacccgccccgaccggagctgagagtaattcatacaaaaggactcgcccctgccttggggaatcccagggaccgtcgttaaactcccactaacgtagaacccagagatcgctgcgttcccgccccctcacccgcccgctctcgtcatcactgaggtggagaatagcatgcgtgaggctccggtgcccgtcagtgggcagagcgcacatcgcccacagtccccgagaagttggggggaggggtcggcaattgaacgggtgcctagagaaggtggcgcggggtaaactgggaaagtgatgtcgtgtactggctccgcctttttcccgagggtgggggagaaccgtatataagtgcagtagtcgccgtgaacgttctttttcgcaacgggtttgccgccagaacacagcgtctcaggggagatctcgtttagtgaaccgtcagatcctcactctcttccgcatcgctgtctgcgagggccagctgttgggctcgcggttgaggacaaactcttcgcggtctttccagtactcttggatcggaaacccgtcggcctccgaacggtactccgccaccgagggacctgagcgagtccgcatcgaccggatcggaaaacctctcgagaaaggcgtctaaccagtcacagtcgcaaggtaggctgagcaccgtggcgggcggcagcgggtggcggtcggggttgtttctggcggaggtgctgctgatgatgtaattaaagtaggcggtcttgagacggcggatggtcgaggtgaggtgtggcaggcttgagatccagctgttggggtgagtactccctctcaaaagcgggcattacttctgcgctaagattgtcagtttccaaaaacgaggaggatttgatattcacctggcccgatctggccatacacttgagtgacaatgacatccactttgcctttctctccacaggtgtccactcccaggtccaagtttaaacgccgccaccatg

SEQ ID NO: 28 - DNA, 1768 bp, Artificial Sequence
  Made in Lab - Polynucleotide cassette 1 full 3'
ctgttctcatcacatcatatcaaggttatataccatcaatattgccacagatgttacttagccttttaatatttctctaatttagtgtatatgcaatgatagttctctgatttctgagattgagtttctcatgtgtaatgattatttagagtttctctttcatctgttcaaatttttgtctagttttattttttactgatttgtaagacttctttttataatctgcatattacaattctctttactggggtgttgcaaatattttctgtcattctatggcctgacttttcttaatggttttttaattttaaaaataagtcttaatattcatgcaatctaattaacaatcttttctttgtggttaggactttgagtcataagaaatttttctctacactgaagtcatgatggcatgcttctatattattttctaaaagatttaaagttttgccttctccatttagacttataattcactggaatttttttgtgtgtatggtatgacatatgggttcccttttattttttacatataaatatatttccctgtttttctaaaaaagaaaaagatcatcattttcccattgtaaaatgccatatttttttcataggtcacttacatatatcaatgggtctgtttctgagctctactctattttatcagcctcactgtctatccccacacatctcatgctttgctctaaatcttgatatttagtggaacattctttcccattttgttctacaagaatatttttgttattgtctttgggctttctatatacattttgaaatgaggttgacaagttacctaggaaaactgtcttcataacaggcctattgattggaaagtttgtcaacgaattgtgggtcttttggggtttgctgccccttttacgcaatgtggatatcctgctttaatgcctttatatgcatgtatacaagcaaaacaggcttttactttctcgccaacttacaaggcctttctcagtaaacagtatatgaccctttaccccgttgctcggcaacggcctggtctgtgccaagtgtttgctgacgcaacccccactggttggggcttggccataggccatcagcgcatgcgtggaacctttgtgtctcctctgccgatccatactgcggaactcctagccgcttgttttgctcgcagcaggtctggagcaaacctcatcgggaccgacaattctgtcgtactctcccgcaagtatacatcgtttccatggctgctaggctgtgctgccaactggatcctgcgcgggacgtcctttgtttacgtcccgtcggcgctgaatcccgcggacgacccctcccggggccgcttggggctctaccgcccgcttctccgtctgccgtaccgtccgaccacggggcgcacctctctttacgcggactccccgtctgtgccttctcatctgccggaccgtgtgcacttcgcttcacctctgcacgtcgcatggaggccaccgtgaacgcccaccggaacctgcccaaggtcttgcataagaggactcttggactttcagcaatgtcatcctgcccgggtggcatccctgtgacccctccccagtgcctctcctggccctggaagttgccactccagtgcccaccagccttgtcctaataaaattaagttgcatcattttgtctgactaggtgtccttctataatattatggggtggaggggggtggtatggagcaaggggcccaagttgggaagaaacctgtagggcctgcgaagacagtcag

SEQ ID NO: 29 - DNA, 1193 bp, Artificial Sequence
  Made in Lab - Polynucleotide cassette 2 full 5'
ctctggagacggcacatcgcccacagtccccgagaagttgggaggggtcggcaattgaaccggtgcctagagaaggtggcgcggggtaaactgggaaagtgatgtcgtgtactggctccgcctttttcccgagggtgggggagaaccgtatataagtgcagtagtcgccgtgaacgttctttttcgcaacgggtttgccgccagaacacaggtaagtgccgtgtgtggttcccgcgggcctggcctctttacgggttatggcccttgcgtgccttgaattacttccacctggctccagtacgtgattcttgatcccgagctggagccaggggcgggccttgcgctttaggagccccttcgcctcgtgcttgagttgaggcctggcctgggcgctggggccgccgcgtgcgaatctggtggcaccttcgcgcctgtctcgctgctttcgataagtctctagccatttaaaatttttgatgacgtgctgcgacgctttttttctggcaagatagtcttgtaaatgcgggccaggatctgcacactggtatttcggtttttgggcccgcggccggcgacggggcccgtgcgtcccagcgcacatgttcggcgaggcggggcctgcgagcgcggccaccgagaatcggacgggggtagtctcaagctggccggcctgctctggtgcctggcctcgcgccgccgtgtatcgccccgccctgggcggcaaggctggcccggtcggcaccagttgcgtgagcggaaagatggccgcttcccggccctgctccagggggctcaaaatggaggacgcggcgctcgggagagcgggcgggtgagtcacccacacaaaggaaaagggcctttccgtcctcagccgtcgcttcatgtgactccacggagtaccgggcgccgtccaggcacctcgattagttctggagcttttggagtacgtcgtctttaggttggggggaggggttttatgcgatggagtttccccacactgagtgggtggagactgaagttaggccagcttggcacttgatgtaattctccttggaatttggcctttttgagtttggatcttggttcattctcaagcctcagacagtggttcaaagtttttttcttccatttcaggtgtcgtgaacacgtctcaggggagatctacacccaagctgtctagagccgccaccatg

SEQ ID NO: 30 - DNA, 984 bp, Artificial Sequence
  Made in Lab - Polynucleotide cassette 2 full 3'
tgaggcatgcttctatattattttctaaaagatttaaagttttgccttctccatttagacttataattcactggaatttttttgtgtgtatggtatgacatatgggttcccttttattttttacatataaatatatttccctgtttttctaaaaaagacctaggaaaactgtcttcataatcaacctctggattacaaaatttgtgaaagattgactggtattcttaactatgttgctccttttacgctatgtggatacgctgctttaatgcctttgtatcatgctattgcttcccgtatggctttcattttctcctccttgtataaatcctggttgctgtctctttatgaggagttgtggcccgttgtcaggcaacgtggcgtggtgtgcactgtgtttgctgacgcaacccccactggttggggcattgccaccacctgtcagctcctttccgggactttcgctttccccctccctattgccacggcggaactcatcgccgcctgccttgcccgctgctggacaggggctcggctgttgggcactgacaattccgtggtgttgtcggggaaatcatcgtcctttccttggctgctcgcctgtgttgccacctggattctgcgcgggacgtccttctgctacgtcccttcggccctcaatccagcggaccttccttcccgcggcctgctgccggctctgcggcctcttccgcctcttcgccttcgccctcagacgagtcggatctccctttgggccgcctccccgcatcctgcccgggtggcatccctgtgacccctccccagtgcctctcctggccctggaagttgccactccagtgcccaccagccttgtcctaataaaattaagttgcatcattttgtctgactaggtgtccttctataatattatggggtggaggggggtggtatggagcaaggggcccaagttgggaagaaacctgtagggcctgcgaagacagtcag

SEQ ID NO: 31 - DNA, 1481 bp, Artificial Sequence
  Made in Lab - Polynucleotide cassette 3 full 5'
ctctggagacgcaacctttggagctaagccagcaatggtagagggaagattctgcacgtcccttccaggcggcctccccgtcaccaccccccccaacccgccccgaccggagctgagagtaattcatacaaaaggactcgcccctgccttggggaatcccagggaccgtcgttaaactcccactaacgtagaacccagagatcgctgcgttcccgccccctcacccgcccgctctcgtcatcactgaggtggagaatagcatgcgtgaggctccggtgcccgtcagtgggcagagcgcacatcgcccacagtccccgagaagttggggggaggggtcggcaattgaacgggtgcctagagaaggtggcgcggggtaaactgggaaagtgatgtcgtgtactggctccgcctttttcccgagggtgggggagaaccgtatataagtgcagtagtcgccgtgaacgttctttttcgcaacgggtttgccgccagaacacaggtaagtgccgtgtgtggttcccgcgggcctggcctctttacgggttatggcccttgcgtgccttgaattacttccacctggctccagtacgtgattcttgatcccgagctggagccaggggcgggccttgcgctttaggagccccttcgcctcgtgcttgagttgaggcctggcctgggcgctggggccgccgcgtgcgaatctggtggcaccttcgcgcctgtctcgctgctttcgataagtctctagccatttaaaatttttgatgacgtgctgcgacgctttttttctggcaagatagtcttgtaaatgcgggccaggatctgcacactggtatttcggtttttgggcccgcggccggcgacggggcccgtgcgtcccagcgcacatgttcggcgaggcggggcctgcgagcgcggccaccgagaatcggacgggggtagtctcaagctggccggcctgctctggtgcctggcctcgcgccgccgtgtatcgccccgccctgggcggcaaggctggcccggtcggcaccagttgcgtgagcggaaagatggccgcttcccggccctgctccagggggctcaaaatggaggacgcggcgctcgggagagcgggcgggtgagtcacccacacaaaggaaaagggcctttccgtcctcagccgtcgcttcatgtgactccacggagtaccgggcgccgtccaggcacctcgattagttctggagcttttggagtacgtcgtctttaggttggggggaggggttttatgcgatggagtttccccacactgagtgggtggagactgaagttaggccagcttggcacttgatgtaattctccttggaatttggcctttttgagtttggatcttggttcattctcaagcctcagacagtggttcaaagtttttttcttccatttcaggtgtcgtgaacacgtctcaggggagatctacacccaagctgtctagagccgccaccatg

SEQ ID NO: 32 - DNA, 581 bp, Artificial Sequence
  Made in Lab - Polynucleotide cassette 3 full 3'
ggttcccttttattttttacatataaatatatttccctgtttttctaaaaaagaaaaagatcatcattttcccattgtaaaatgccatatttttttcataggtcacttacatatatcaatgggtctgtttctgagctctactctattttatcagcctcactgtctatccccacacatctcatgctttgctctaaatcttgatatttagtggaacattctttcccattttgttctacaagaatatttttgttattgtctttgggctttctatatacattttgaaatgaggttgacaagttacctaggaaaactgtcttcttgccagccatctgttgtttgcccctcccccgtgccttccttgaccctggaaggtgccactcccactgtcctttcctaataaaatgaggaaattgcatcgcattgtctgagtaggtgtcattctattctggggggtggggtggggcaggacagcaagggggaggattgggaatacaatagcaggcatgctggggatgcggtgggctctatgggtacccaggtgctgaagaattgacccggttcctcctggggaagacagtcag

SEQ ID NO: 33 - DNA, 1511 bp, Artificial Sequence
  Made in Lab - Polynucleotide cassette 4 full 5'
ctctggagacgcaacctttggagctaagccagcaatggtagagggaagattctgcacgtcccttccaggcggcctccccgtcaccaccccccccaacccgccccgaccggagctgagagtaattcatacaaaaggactcgcccctgccttggggaatcccagggaccgtcgttaaactcccactaacgtagaacccagagatcgctgcgttcccgccccctcacccgcccgctctcgtcatcactgaggtggagaatagcatgcgtgaggctccggtgcccgtcagtgggcagagcgcacatcgcccacagtccccgagaagttggggggaggggtcggcaattgaacgggtgcctagagaaggtggcgcggggtaaactgggaaagtgatgtcgtgtactggctccgcctttttcccgagggtgggggagaaccgtatataagtgcagtagtcgccgtgaacgttctttttcgcaacgggtttgccgccagaacacaggtaagtgccgtgtgtggttcccgcgggcctggcctctttacgggttatggcccttgcgtgccttgaattacttccacctggctccagtacgtgattcttgatcccgagctggagccaggggcgggccttgcgctttaggagccccttcgcctcgtgcttgagttgaggcctggcctgggcgctggggccgccgcgtgcgaatctggtggcaccttcgcgcctgtctcgctgctttcgataagtctctagccatttaaaatttttgatgacgtgctgcgacgctttttttctggcaagatagtcttgtaaatgcgggccaggatctgcacactggtatttcggtttttgggcccgcggccggcgacggggcccgtgcgtcccagcgcacatgttcggcgaggcggggcctgcgagcgcggccaccgagaatcggacgggggtagtctcaagctggccggcctgctctggtgcctggcctcgcgccgccgtgtatcgccccgccctgggcggcaaggctggcccggtcggcaccagttgcgtgagcggaaagatggccgcttcccggccctgctccagggggctcaaaatggaggacgcggcgctcgggagagcgggcgggtgagtcacccacacaaaggaaaagggcctttccgtcctcagccgtcgcttcatgtgactccacggagtaccgggcgccgtccaggcacctcgattagttctggagcttttggagtacgtcgtctttaggttggggggaggggttttatgcgatggagtttccccacactgagtgggtggagactgaagttaggccagcttggcacttgatgtaattctccttggaatttggcctttttgagtttggatcttggttcattctcaagcctcagacagtggttcaaagtttttttcttccatttcaggtgtcgtgaacacgtctcaggggagatctagcttgcttgttctttttgcagaagctcagaataaacgctcaactttggccgccaccatg

SEQ ID NO: 34 - DNA, 717 bp, Artificial Sequence
  Made in Lab - Polynucleotide cassette 4 full 3'
ggttcccttttattttttacatataaatatatttccctgtttttctaaaaaagaaaaagatcatcattttcccattgtaaaatgccatatttttttcataggtcacttacatatatcaatgggtctgtttctgagctctactctattttatcagcctcactgtctatccccacacatctcatgctttgctctaaatcttgatatttagtggaacattctttcccattttgttctacaagaatatttttgttattgtctttgggctttctatatacattttgaaatgaggttgacaagttacctaggaaaactgtcttctggctaataaaggaaatttattttcattgcaatagtgtgttggaattttttgtgtctctcactcggaaggacatatgggagggcaaatcatttaaaacatcagaatgagtatttggtttagagtttggcaacatatgcccatatgctggctgccatgaacaaaggttggctataaagaggtcatcagtatatgaaacagccccctgctgtccattccttattccatagaaaagccttgacttgaggttagattttttttatattttgttttgtgttatttttttctttaacatccctaaaattttccttacatgttttactagccagatttttcctcctctcctgactactcccagtcatagctgtccctcttctcttatggagatcgaagacagtcag

SEQ ID NO: 35 - DNA, 928 bp, Artificial Sequence
  Made in Lab - Polynucleotide cassette 5 full 5'
ctctggagacgacttacggtaaatggcccgcctggctgaccgcccaacgacccccgcccattgacgtcaataatgacgtatgttcccatagtaacgccaatagggactttccattgacgtcaatgggtggagtatttacggtaaactgcccacttggcagtacatcaagtgtatcatatgccaagtccgccccctattgacgtcaatgacggtaaatggcccgcctggcattatgcccagtacatgaccttacgggactttcctacttggcagtacatctacgtattagtcatcgctattaccaatgacgtcgaggagaagttccccaactttcccgcctctcagcctttgaaagaaagaaaggggagggggcaggccgcgtgcagccgcgagcggtgctgggctccggctccaattccccatctcagtcgttcccaaagtcctcctgtttcatccaagcgtgtaagggtccccgtccttgactccctagtgtcctgctgcccacagtccagtcctgggaaccagcaccgatcacctcccatcgggccaatctcagtcccttcccccctacgtcggggcccacacgctcggtgcgtgcccagttgaaccaggcggctgcggaaaaaaaaaagcggggagaaagtagggcccggctactagcggttttacgggcgcacgtagctcaggcctcaagaccttgggctgggactggctgagcctggcgggaggcggggtccgagtcaccgcctgccgccgcgcccccggtttctataaattgagcccgcagcctcccgcttcgctctctgctcctcctgttcgacagtcagccgcatcttcttttgcgtcgccagcgtctcaggggagatctagcttgcttgttctttttgcagaagctcagaataaacgctcaactttggccgccaccatg

SEQ ID NO: 36 - DNA, 1268 bp, Artificial Sequence
  Made in Lab - Polynucleotide cassette 5 full 3'
ggttcccttttattttttacatataaatatatttccctgtttttctaaaaaagaaaaagatcatcattttcccattgtaaaatgccatatttttttcataggtcacttacatatatcaatgggtctgtttctgagctctactctattttatcagcctcactgtctatccccacacatctcatgctttgctctaaatcttgatatttagtggaacattctttcccattttgttctacaagaatatttttgttattgtctttgggctttctatatacattttgaaatgaggttgacaagttacctaggaaaactgtcttcataacaggcctattgattggaaagtttgtcaacgaattgtgggtcttttggggtttgctgccccttttacgcaatgtggatatcctgctttaatgcctttatatgcatgtatacaagcaaaacaggcttttactttctcgccaacttacaaggcctttctcagtaaacagtatatgaccctttaccccgttgctcggcaacggcctggtctgtgccaagtgtttgctgacgcaacccccactggttggggcttggccataggccatcagcgcatgcgtggaacctttgtgtctcctctgccgatccatactgcggaactcctagccgcttgttttgctcgcagcaggtctggagcaaacctcatcgggaccgacaattctgtcgtactctcccgcaagtatacatcgtttccatggctgctaggctgtgctgccaactggatcctgcgcgggacgtcctttgtttacgtcccgtcggcgctgaatcccgcggacgacccctcccggggccgcttggggctctaccgcccgcttctccgtctgccgtaccgtccgaccacggggcgcacctctctttacgcggactccccgtctgtgccttctcatctgccggaccgtgtgcacttcgcttcacctctgcacgtcgcatggaggccaccgtgaacgcccaccggaacctgcccaaggtcttgcataagaggactcttggactttcagcaatgtcatcctgcccgggtggcatccctgtgacccctccccagtgcctctcctggccctggaagttgccactccagtgcccaccagccttgtcctaataaaattaagttgcatcattttgtctgactaggtgtccttctataatattatggggtggaggggggtggtatggagcaaggggcccaagttgggaagaaacctgtagggcctgcgaagacagtcagactgtcatta

SEQ ID NO: 37 - DNA, 1427 bp, Artificial Sequence
  Made in Lab - Polynucleotide cassette 6 full 5'
ctctggagacgacttacggtaaatggcccgcctggctgaccgcccaacgacccccgcccattgacgtcaataatgacgtatgttcccatagtaacgccaatagggactttccattgacgtcaatgggtggagtatttacggtaaactgcccacttggcagtacatcaagtgtatcatatgccaagtccgccccctattgacgtcaatgacggtaaatggcccgcctggcattatgcccagtacatgaccttacgggactttcctacttggcagtacatctacgtattagtcatcgctattaccaatgacgtcgaggagaagttccccaactttcccgcctctcagcctttgaaagaaagaaaggggagggggcaggccgcgtgcagccgcgagcggtgctgggctccggctccaattccccatctcagtcgttcccaaagtcctcctgtttcatccaagcgtgtaagggtccccgtccttgactccctagtgtcctgctgcccacagtccagtcctgggaaccagcaccgatcacctcccatcgggccaatctcagtcccttcccccctacgtcggggcccacacgctcggtgcgtgcccagttgaaccaggcggctgcggaaaaaaaaaagcggggagaaagtagggcccggctactagcggttttacgggcgcacgtagctcaggcctcaagaccttgggctgggactggctgagcctggcgggaggcggggtccgagtcaccgcctgccgccgcgcccccggtttctataaattgagcccgcagcctcccgcttcgctctctgctcctcctgttcgacagtcagccgcatcttcttttgcgtcgccagcgtctcaggggagatctcgtttagtgaaccgtcagatcctcactctcttccgcatcgctgtctgcgagggccagctgttgggctcgcggttgaggacaaactcttcgcggtctttccagtactcttggatcggaaacccgtcggcctccgaacggtactccgccaccgagggacctgagcgagtccgcatcgaccggatcggaaaacctctcgagaaaggcgtctaaccagtcacagtcgcaaggtaggctgagcaccgtggcgggcggcagcgggtggcggtcggggttgtttctggcggaggtgctgctgatgatgtaattaaagtaggcggtcttgagacggcggatggtcgaggtgaggtgtggcaggcttgagatccagctgttggggtgagtactccctctcaaaagcgggcattacttctgcgctaagattgtcagtttccaaaaacgaggaggatttgatattcacctggcccgatctggccatacacttgagtgacaatgacatccactttgcctttctctccacaggtgtccactcccaggtccaagtttaaacgccgccaccatg

SEQ ID NO: 38 - DNA, 1169 bp, Artificial Sequence
  Made in Lab - Polynucleotide cassette 6 full 3'
tgaggcatgcttctatattattttctaaaagatttaaagttttgccttctccatttagacttataattcactggaatttttttgtgtgtatggtatgacatatgggttcccttttattttttacatataaatatatttccctgtttttctaaaaaagacctaggaaaactgtcttcataatcaacctctggattacaaaatttgtgaaagattgactggtattcttaactatgttgctccttttacgctatgtggatacgctgctttaatgcctttgtatcatgctattgcttcccgtatggctttcattttctcctccttgtataaatcctggttgctgtctctttatgaggagttgtggcccgttgtcaggcaacgtggcgtggtgtgcactgtgtttgctgacgcaacccccactggttggggcattgccaccacctgtcagctcctttccgggactttcgctttccccctccctattgccacggcggaactcatcgccgcctgccttgcccgctgctggacaggggctcggctgttgggcactgacaattccgtggtgttgtcggggaaatcatcgtcctttccttggctgctcgcctgtgttgccacctggattctgcgcgggacgtccttctgctacgtcccttcggccctcaatccagcggaccttccttcccgcggcctgctgccggctctgcggcctcttccgcctcttcgccttcgccctcagacgagtcggatctccctttgggccgcctccccgcatctggctaataaaggaaatttattttcattgcaatagtgtgttggaattttttgtgtctctcactcggaaggacatatgggagggcaaatcatttaaaacatcagaatgagtatttggtttagagtttggcaacatatgcccatatgctggctgccatgaacaaaggttggctataaagaggtcatcagtatatgaaacagccccctgctgtccattccttattccatagaaaagccttgacttgaggttagattttttttatattttgttttgtgttatttttttctttaacatccctaaaattttccttacatgttttactagccagatttttcctcctctcctgactactcccagtcatagctgtccctcttctcttatggagatcgaagacagtcag

SEQ ID NO: 39 - DNA, 1755 bp, Artificial Sequence
  Made in Lab - Polynucleotide cassette 7 full 5'
ctctggagacgcgttacataacttacggtaaatggcccgcctggctgaccgcccaacgacccccgcccattgacgtcaataatgacgtatgttcccatagtaacgccaatagggactttccattgacgtcaatgggtggagtatttacggtaaactgcccacttggcagtacatcaagtgtatcatatgccaagtacgccccctattgacgtcaatgacggtaaatggcccgcctggcattatgcccagtacatgaccttatgggactttcctacttggcagtacatctacgtattagtcatcgctattaccatggtcgaggtgagccccacgttctgcttcactctccccatctcccccccctccccacccccaattttgtatttatttattttttaattattttgtgcagcgatgggggcggggggggggggggcgcgcgccaggcggggcggggcggggcgaggggcggggcggggcgaggcggagaggtgcggcggcagccaatcagagcggcgcgctccgaaagtttccttttatggcgaggcggcggcggcggcggccctataaaaagcgaagcgcgcggcgggcgggagtcgctgcgcgctgccttcgccccgtgccccgctccgccgccgcctcgcgccgcccgccccggctctgactgaccgcgttactcccacaggtgagcgggcgggacggcccttctcctccgggctgtaattagcgcttggtttaatgacggcttgtttcttttctgtggctgcgtgaaagccttgaggggctccgggagggccctttgtgcgggggggagcggctcggggggtgcgtgcgtgtgtgtgtgcgtggggagcgccgcgtgcggctccgcgctgcccggcggctgtgagcgctgcgggcgcggcgcggggctttgtgcgctccgcagtgtgcgcgaggggagcgcggccgggggcggtgccccgcggtgcggggggggctgcgaggggaacaaaggctgcgtgcggggtgtgtgcgtgggggggtgagcagggggtgtgggcgcgtcggtcgggctgcaaccccccctgcacccccctccccgagttgctgagcacggcccggcttcgggtgcggggctccgtacggggcgtggcgcggggctcgccgtgccgggcggggggtggcggcaggtgggggtgccgggcggggcggggccgcctcgggccggggagggctcgggggaggggcgcggcggcccccggagcgccggcggctgtcgaggcgcggcgagccgcagccattgccttttatggtaatcgtgcgagagggcgcagggacttcctttgtcccaaatctgtgcggagccgaaatctgggaggcgccgccgcaccccctctagcgggcgcggggcgaagcggtgcggcgccggcaggaaggaaatgggcggggagggccttcgtgcgtcgccgcgccgccgtccccttctccctctccagcctcggggctgtccgcggggggacggctgccttcgggggggacggggcagggcggggttcggcttctggcgtgtgaccggcggctctagagcctctgctaaccatgttcatgccttcttctttttcctacagctcctgggcaacgtgctggttattgtgctgtctcatcattttggcaaagaattcggcttgatcgaagccgtctcaggggagatctagcttgcttgttctttttgcagaagctcagaataaacgctcaactttggccgccaccatg

SEQ ID NO: 40 - DNA, 1165 bp, Artificial Sequence
  Made in Lab - Polynucleotide cassette 7 full 3'
tgaggcatgcttctatattattttctaaaagatttaaagttttgccttctccatttagacttataattcactggaatttttttgtgtgtatggtatgacatatgggttcccttttattttttacatataaatatatttccctgtttttctaaaaaagacctaggaaaactgtcttcataacaggcctattgattggaaagtttgtcaacgaattgtgggtcttttggggtttgctgccccttttacgcaatgtggatatcctgctttaatgcctttatatgcatgtatacaagcaaaacaggcttttactttctcgccaacttacaaggcctttctcagtaaacagtatatgaccctttaccccgttgctcggcaacggcctggtctgtgccaagtgtttgctgacgcaacccccactggttggggcttggccataggccatcagcgcatgcgtggaacctttgtgtctcctctgccgatccatactgcggaactcctagccgcttgttttgctcgcagcaggtctggagcaaacctcatcgggaccgacaattctgtcgtactctcccgcaagtatacatcgtttccatggctgctaggctgtgctgccaactggatcctgcgcgggacgtcctttgtttacgtcccgtcggcgctgaatcccgcggacgacccctcccggggccgcttggggctctaccgcccgcttctccgtctgccgtaccgtccgaccacggggcgcacctctctttacgcggactccccgtctgtgccttctcatctgccggaccgtgtgcacttcgcttcacctctgcacgtcgcatggaggccaccgtgaacgcccaccggaacctgcccaaggtcttgcataagaggactcttggactttcagcaatgtcatcttgccagccatctgttgtttgcccctcccccgtgccttccttgaccctggaaggtgccactcccactgtcctttcctaataaaatgaggaaattgcatcgcattgtctgagtaggtgtcattctattctggggggtggggtggggcaggacagcaagggggaggattgggaatacaatagcaggcatgctggggatgcggtgggctctatgggtacccaggtgctgaagaattgacccggttcctcctggggaagacagtcag

SEQ ID NO: 41 - DNA, 1159 bp, Artificial Sequence
  Made in Lab - Polynucleotide cassette 8 full 5'
ctctggagacgacttacggtaaatggcccgcctggctgaccgcccaacgacccccgcccattgacgtcaataatgacgtatgttcccatagtaacgccaatagggactttccattgacgtcaatgggtggagtatttacggtaaactgcccacttggcagtacatcaagtgtatcatatgccaagtccgccccctattgacgtcaatgacggtaaatggcccgcctggcattatgcccagtacatgaccttacgggactttcctacttggcagtacatctacgtattagtcatcgctattaccatggtcgaggtgagccccacgttctgcttcactctccccatctcccccccctccccacccccaattttgtatttatttattttttaattattttgtgcagcgatgggggcgggggggggggggcgcgcgccaggcggggcggggcggggcgaggggcggggcggggcgaggcggagaggtgcggcggcagccaatcagagcggcgcgctccgaaagtttccttttatggcgaggcggcggcggcggcggccctataaaaagcgaagcgcgcggcgggcggcgtctcaggggagatctcgtttagtgaaccgtcagatcctcactctcttccgcatcgctgtctgcgagggccagctgttgggctcgcggttgaggacaaactcttcgcggtctttccagtactcttggatcggaaacccgtcggcctccgaacggtactccgccaccgagggacctgagcgagtccgcatcgaccggatcggaaaacctctcgagaaaggcgtctaaccagtcacagtcgcaaggtaggctgagcaccgtggcgggcggcagcgggtggcggtcggggttgtttctggcggaggtgctgctgatgatgtaattaaagtaggcggtcttgagacggcggatggtcgaggtgaggtgtggcaggcttgagatccagctgttggggtgagtactccctctcaaaagcgggcattacttctgcgctaagattgtcagtttccaaaaacgaggaggatttgatattcacctggcccgatctggccatacacttgagtgacaatgacatccactttgcctttctctccacaggtgtccactcccaggtccaagtttaaacgccgccaccatg

SEQ ID NO: 42 - DNA, 572 bp, Artificial Sequence
  Made in Lab - Polynucleotide cassette 8 full 3'
ggcatgcttctatattattttctaaaagatttaaagttttgccttctccatttagacttataattcactggaatttttttgtgtgtatggtatgacatatgggttcccttttattttttacatataaatatatttccctgtttttctaaaaaagacctaggaaaactgtcttctggctaataaaggaaatttattttcattgcaatagtgtgttggaattttttgtgtctctcactcggaaggacatatgggagggcaaatcatttaaaacatcagaatgagtatttggtttagagtttggcaacatatgcccatatgctggctgccatgaacaaaggttggctataaagaggtcatcagtatatgaaacagccccctgctgtccattccttattccatagaaaagccttgacttgaggttagattttttttatattttgttttgtgttatttttttctttaacatccctaaaattttccttacatgttttactagccagatttttcctcctctcctgactactcccagtcatagctgtccctcttctcttatggagatcgaagacagtcag

SEQ ID NO: 43 - DNA, 1519 bp, Artificial Sequence
  Made in Lab - Polynucleotide cassette 9 full 5'
ctctggagacgacttacggtaaatggcccgcctggctgaccgcccaacgacccccgcccattgacgtcaataatgacgtatgttcccatagtaacgccaatagggactttccattgacgtcaatgggtggagtatttacggtaaactgcccacttggcagtacatcaagtgtatcatatgccaagtccgccccctattgacgtcaatgacggtaaatggcccgcctggcattatgcccagtacatgaccttacgggactttcctacttggcagtacatctacgtattagtcatcgctattaccagcacatcgcccacagtccccgagaagttggggggaggggtcggcaattgaaccggtgcctagagaaggtggcgcggggtaaactgggaaagtgatgtcgtgtactggctccgcctttttcccgagggtgggggagaaccgtatataagtgcagtagtcgccgtgaacgttctttttcgcaacgggtttgccgccagaacacaggtaagtgccgtgtgtggttcccgcgggcctggcctctttacgggttatggcccttgcgtgccttgaattacttccacctggctccagtacgtgattcttgatcccgagctggagccaggggcgggccttgcgctttaggagccccttcgcctcgtgcttgagttgaggcctggcctgggcgctggggccgccgcgtgcgaatctggtggcaccttcgcgcctgtctcgctgctttcgataagtctctagccatttaaaatttttgatgacgtgctgcgacgctttttttctggcaagatagtcttgtaaatgcgggccaggatctgcacactggtatttcggtttttgggcccgcggccggcgacggggcccgtgcgtcccagcgcacatgttcggcgaggcggggcctgcgagcgcggccaccgagaatcggacgggggtagtctcaagctggccggcctgctctggtgcctggcctcgcgccgccgtgtatcgccccgccctgggcggcaaggctggcccggtcggcaccagttgcgtgagcggaaagatggccgcttcccggccctgctccagggggctcaaaatggaggacgcggcgctcgggagagcgggcgggtgagtcacccacacaaaggaaaagggcctttccgtcctcagccgtcgcttcatgtgactccacggagtaccgggcgccgtccaggcacctcgattagttctggagcttttggagtacgtcgtctttaggttggggggaggggttttatgcgatggagtttccccacactgagtgggtggagactgaagttaggccagcttggcacttgatgtaattctccttggaatttggcctttttgagtttggatcttggttcattctcaagcctcagacagtggttcaaagtttttttcttccatttcaggtgtcctgaacacgtctcaggggagatctagcttgcttgttctttttgcagaagctcagaataaacgctcaactttggccgccaccatg

SEQ ID NO: 44 - DNA, 387 bp, Artificial Sequence
  Made in Lab - Polynucleotide cassette 9 full 3'
ggcatgcttctatattattttctaaaagatttaaagttttgccttctccatttagacttataattcactggaatttttttgtgtgtatggtatgacatatgggttcccttttattttttacatataaatatatttccctgtttttctaaaaaagacctaggaaaactgtcttcctgcccgggtggcatccctgtgacccctccccagtgcctctcctggccctggaagttgccactccagtgcccaccagccttgtcctaataaaattaagttgcatcattttgtctgactaggtgtccttctataatattatggggtggaggggggtggtatggagcaaggggcccaagttgggaagaaacctgtagggcctgcgaagacagtcag

SEQ ID NO: 45 - DNA, 1489 bp, Artificial Sequence
  Made in Lab - Polynucleotide cassette 10 full 5'
ctctggagacgacttacggtaaatggcccgcctggctgaccgcccaacgacccccgcccattgacgtcaataatgacgtatgttcccatagtaacgccaatagggactttccattgacgtcaatgggtggagtatttacggtaaactgcccacttggcagtacatcaagtgtatcatatgccaagtccgccccctattgacgtcaatgacggtaaatggcccgcctggcattatgcccagtacatgaccttacgggactttcctacttggcagtacatctacgtattagtcatcgctattaccagcacatcgcccacagtccccgagaagttggggggaggggtcggcaattgaaccggtgcctagagaaggtggcgcggggtaaactgggaaagtgatgtcgtgtactggctccgcctttttcccgagggtgggggagaaccgtatataagtgcagtagtcgccgtgaacgttctttttcgcaacgggtttgccgccagaacacaggtaagtgccgtgtgtggttcccgcgggcctggcctctttacgggttatggcccttgcgtgccttgaattacttccacctggctccagtacgtgattcttgatcccgagctggagccaggggcgggccttgcgctttaggagccccttcgcctcgtgcttgagttgaggcctggcctgggcgctggggccgccgcgtgcgaatctggtggcaccttcgcgcctgtctcgctgctttcgataagtctctagccatttaaaatttttgatgacgtgctgcgacgctttttttctggcaagatagtcttgtaaatgcgggccaggatctgcacactggtatttcggtttttgggcccgcggccggcgacggggcccgtgcgtcccagcgcacatgttcggcgaggcggggcctgcgagcgcggccaccgagaatcggacgggggtagtctcaagctggccggcctgctctggtgcctggcctcgcgccgccgtgtatcgccccgccctgggcggcaaggctggcccggtcggcaccagttgcgtgagcggaaagatggccgcttcccggccctgctccagggggctcaaaatggaggacgcggcgctcgggagagcgggcgggtgagtcacccacacaaaggaaaagggcctttccgtcctcagccgtcgcttcatgtgactccacggagtaccgggcgccgtccaggcacctcgattagttctggagcttttggagtacgtcgtctttaggttggggggaggggttttatgcgatggagtttccccacactgagtgggtggagactgaagttaggccagcttggcacttgatgtaattctccttggaatttggcctttttgagtttggatcttggttcattctcaagcctcagacagtggttcaaagtttttttcttccatttcaggtgtcctgaacacgtctcaggggagatctacacccaagctgtctagagccgccaccatg

SEQ ID NO: 46 - DNA, 1180 bp, Artificial Sequence
  Made in Lab - Polynucleotide cassette 10 full 3'
ggttcccttttattttttacatataaatatatttccctgtttttctaaaaaagaaaaagatcatcattttcccattgtaaaatgccatatttttttcataggtcacttacatatatcaatgggtctgtttctgagctctactctattttatcagcctcactgtctatccccacacatctcatgctttgctctaaatcttgatatttagtggaacattctttcccattttgttctacaagaatatttttgttattgtctttgggctttctatatacattttgaaatgaggttgacaagttacctaggaaaactgtcttcatataatcaacctctggattacaaaatttgtgaaagattgactggtattcttaactatgttgctccttttacgctatgtggatacgctgctttaatgcctttgtatcatgctattgcttcccgtatggctttcattttctcctccttgtataaatcctggttgctgtctctttatgaggagttgtggcccgttgtcaggcaacgtggcgtggtgtgcactgtgtttgctgacgcaacccccactggttggggcattgccaccacctgtcagctcctttccgggactttcgctttccccctccctattgccacggcggaactcatcgccgcctgccttgcccgctgctggacaggggctcggctgttgggcactgacaattccgtggtgttgtcggggaaatcatcgtcctttccttggctgctcgcctgtgttgccacctggattctgcgcgggacgtccttctgctacgtcccttcggccctcaatccagcggaccttccttcccgcggcctgctgccggctctgcggcctcttccgcctcttcgccttcgccctcagacgagtcggatctccctttgggccgcctccccgcatcatcttgccagccatctgttgtttgcccctcccccgtgccttccttgaccctggaaggtgccactcccactgtcctttcctaataaaatgaggaaattgcatcgcattgtctgagtaggtgtcattctattctggggggtggggtggggcaggacagcaagggggaggattgggaatacaatagcaggcatgctggggatgcggtgggctctatgggtacccaggtgctgaagaattgacccggttcctcctggggaagacagtcag

SEQ ID NO: 47 - DNA, 1172 bp, Artificial Sequence
  Made in Lab - Polynucleotide cassette 11 full 5'
ctctggagacgacttacggtaaatggcccgcctggctgaccgcccaacgacccccgcccattgacgtcaataatgacgtatgttcccatagtaacgccaatagggactttccattgacgtcaatgggtggagtatttacggtaaactgcccacttggcagtacatcaagtgtatcatatgccaagtccgccccctattgacgtcaatgacggtaaatggcccgcctggcattatgcccagtacatgaccttacgggactttcctacttggcagtacatctacgtattagtcatcgctattaccatgctgatgcggttttggcagtacaccaatgggcgtggatagcggtttgactcacggggatttccaagtctccaccccattgacgtcaatgggagtttgttttggcaccaaaatcaacgggactttccaaaatgtcgtaataaccccgccccgttgacgcaaatgggcggtaggcgtgtacggtgggaggtctatataagcagagctcgtttagtgaaccgtcagatcgcctggagaggccatccacgctgttttgacctccatagtggacaccgggaccgatccagcctccgcgtctcaggggagatctcgtttagtgaaccgtcagatcctcactctcttccgcatcgctgtctgcgagggccagctgttgggctcgcggttgaggacaaactcttcgcggtctttccagtactcttggatcggaaacccgtcggcctccgaacggtactccgccaccgagggacctgagcgagtccgcatcgaccggatcggaaaacctctcgagaaaggcgtctaaccagtcacagtcgcaaggtaggctgagcaccgtggcgggcggcagcgggtggcggtcggggttgtttctggcggaggtgctgctgatgatgtaattaaagtaggcggtcttgagacggcggatggtcgaggtgaggtgtggcaggcttgagatccagctgttggggtgagtactccctctcaaaagcgggcattacttctgcgctaagattgtcagtttccaaaaacgaggaggatttgatattcacctggcccgatctggccatacacttgagtgacaatgacatccactttgcctttctctccacaggtgtccactcccaggtccaagtttaaacgccgccaccatg

SEQ ID NO: 48 - DNA, 1043 bp, Artificial Sequence
  Made in Lab - Polynucleotide cassette 11 full 3'
actgttctcatcacatcatatcaaggttatataccatcaatattgccacagatgttacttagccttttaatatttctctaatttagtgtatatgcaatgatagttctctgatttctgagattgagtttctcatgtgtaatgattatttagagtttctctttcatctgttcaaatttttgtctagttttattttttactgatttgtaagacttctttttataatctgcatattacaattctctttactggggtgttgcaaatattttctgtcattctatggcctgacttttcttaatggttttttaattttaaaaataagtcttaatattcatgcaatctaattaacaatcttttctttgtggttaggactttgagtcataagaaatttttctctacactgaagtcatgatggcatgcttctatattattttctaaaagatttaaagttttgccttctccatttagacttataattcactggaatttttttgtgtgtatggtatgacatatgggttcccttttattttttacatataaatatatttccctgtttttctaaaaaagaaaaagatcatcattttcccattgtaaaatgccatatttttttcataggtcacttacatatatcaatgggtctgtttctgagctctactctattttatcagcctcactgtctatccccacacatctcatgctttgctctaaatcttgatatttagtggaacattctttcccattttgttctacaagaatatttttgttattgtctttgggctttctatatacattttgaaatgaggttgacaagttacctaggaaaactgtcttcctgcccgggtggcatccctgtgacccctccccagtgcctctcctggccctggaagttgccactccagtgcccaccagccttgtcctaataaaattaagttgcatcattttgtctgactaggtgtccttctataatattatggggtggaggggggtggtatggagcaaggggcccaagttgggaagaaacctgtagggcctgcgaagacagtcag

SEQ ID NO: 49 - DNA, 1172 bp, Artificial Sequence; identical to SEQ ID NO: 47
  Made in Lab - Polynucleotide cassette 12 full 5'

SEQ ID NO: 50 - DNA, 1165 bp, Artificial Sequence; identical to SEQ ID NO: 40
  Made in Lab - Polynucleotide cassette 12 full 3'

SEQ ID NO: 51 - DNA, 820 bp, Artificial Sequence
  Made in Lab - Polynucleotide cassette 13 full 5'
ctctggagacgacttacggtaaatggcccgcctggctgaccgcccaacgacccccgcccattgacgtcaataatgacgtatgttcccatagtaacgccaatagggactttccattgacgtcaatgggtggagtatttacggtaaactgcccacttggcagtacatcaagtgtatcatatgccaagtccgccccctattgacgtcaatgacggtaaatggcccgcctggcattatgcccagtacatgaccttacgggactttcctacttggcagtacatctacgtattagtcatcgctattaccatggtcgaggtgagccccacgttctgcttcactctccccatctcccccccctccccacccccaattttgtatttatttattttttaattattttgtgcagcgatgggggcgggggggggggggcgcgcgccaggcggggcggggcggggcgaggggcggggcggggcgaggcggagaggtgcggcggcagccaatcagagcggcgcgctccgaaagtttccttttatggcgaggcggcggcggcggcggccctataaaaagcgaagcgcgcggcgggcggcgtctcaggggagatctggtgaggtgtggcaggcttgagatccagctgttggggtgagtactccctctcaaaagcgggcattacttctgcgctaagattgtcagtttccaaaaacgaggaggatttgatattcacctggcccgatctggccatacacttgagtgacaatgacatccactttgcctttctctccacaggtgtccactcccaggtccaagtttaaacgccgccaccatg

SEQ ID NO: 52 - DNA, 1443 bp, Artificial Sequence
  Made in Lab - Polynucleotide cassette 13 full 3'
ggttcccttttattttttacatataaatatatttccctgtttttctaaaaaagaaaaagatcatcattttcccattgtaaaatgccatatttttttcataggtcacttacatatatcaatgggtctgtttctgagctctactctattttatcagcctcactgtctatccccacacatctcatgctttgctctaaatcttgatatttagtggaacattctttcccattttgttctacaagaatatttttgttattgtctttgggctttctatatacattttgaaatgaggttgacaagttacctaggaaaactgtcttcataacaggcctattgattggaaagtttgtcaacgaattgtgggtcttttggggtttgctgccccttttacgcaatgtggatatcctgctttaatgcctttatatgcatgtatacaagcaaaacaggcttttactttctcgccaacttacaaggcctttctcagtaaacagtatatgaccctttaccccgttgctcggcaacggcctggtctgtgccaagtgtttgctgacgcaacccccactggttggggcttggccataggccatcagcgcatgcgtggaacctttgtgtctcctctgccgatccatactgcggaactcctagccgcttgttttgctcgcagcaggtctggagcaaacctcatcgggaccgacaattctgtcgtactctcccgcaagtatacatcgtttccatggctgctaggctgtgctgccaactggatcctgcgcgggacgtcctttgtttacgtcccgtcggcgctgaatcccgcggacgacccctcccggggccgcttggggctctaccgcccgcttctccgtctgccgtaccgtccgaccacggggcgcacctctctttacgcggactccccgtctgtgccttctcatctgccggaccgtgtgcacttcgcttcacctctgcacgtcgcatggaggccaccgtgaacgcccaccggaacctgcccaaggtcttgcataagaggactcttggactttcagcaatgtcatctggctaataaaggaaatttattttcattgcaatagtgtgttggaattttttgtgtctctcactcggaaggacatatgggagggcaaatcatttaaaacatcagaatgagtatttggtttagagtttggcaacatatgcccatatgctggctgccatgaacaaaggttggctataaagaggtcatcagtatatgaaacagccccctgctgtccattccttattccatagaaaagccttgacttgaggttagattttttttatattttgttttgtgttatttttttctttaacatccctaaaattttccttacatgttttactagccagatttttcctcctctcctgactactcccagtcatagctgtccctcttctcttatggagatcgaagacagtcag

SEQ ID NO: 53 - DNA, 920 bp, Artificial Sequence
  Made in Lab - Polynucleotide cassette 14 full 5'
ctctggagacgacttacggtaaatggcccgcctggctgaccgcccaacgacccccgcccattgacgtcaataatgacgtatgttcccatagtaacgccaatagggactttccattgacgtcaatgggtggagtatttacggtaaactgcccacttggcagtacatcaagtgtatcatatgccaagtccgccccctattgacgtcaatgacggtaaatggcccgcctggcattatgcccagtacatgaccttacgggactttcctacttggcagtacatctacgtattagtcatcgctattaccatgctgatgcggttttggcagtacaccaatgggcgtggatagcggtttgactcacggggatttccaagtctccaccccattgacgtcaatgggagtttgttttggcaccaaaatcaacgggactttccaaaatgtcgtaataaccccgccccgttgacgcaaatgggcggtaggcgtgtacggtgggaggtctatataagcagagctcgtttagtgaaccgtcagatcgcctggagaggccatccacgctgttttgacctccatagtggacaccgggaccgatccagcctccgcggccgggaacggtgcattggaacgcggattccccgtgccaagagtgaccctggcagaactcggtaagtctgttgacatgtatgtgatgtatactaacctgcatgggacgtggatttacttgtgtatgtcagatagagtaaagattaactcttgcatgtgagcggggcatcgagatagcgataaatgagtcaggaggacggatacttatatgtgttgttatcctcctctacagtcaaacagattaagcgtctcaggggagatctagcttgcttgttctttttgcagaagctcagaataaacgctcaactttggccgccaccatg

SEQ ID NO: 54 - DNA, 1821 bp, Artificial Sequence
  Made in Lab - Polynucleotide cassette 14 full 3'
ctgttctcatcacatcatatcaaggttatataccatcaatattgccacagatgttacttagccttttaatatttctctaatttagtgtatatgcaatgatagttctctgatttctgagattgagtttctcatgtgtaatgattatttagagtttctctttcatctgttcaaatttttgtctagttttattttttactgatttgtaagacttctttttataatctgcatattacaattctctttactggggtgttgcaaatattttctgtcattctatggcctgacttttcttaatggttttttaattttaaaaataagtcttaatattcatgcaatctaattaacaatcttttctttgtggttaggactttgagtcataagaaatttttctctacactgaagtcatgatggcatgcttctatattattttctaaaagatttaaagttttgccttctccatttagacttataattcactggaatttttttgtgtgtatggtatgacatatgggttcccttttattttttacatataaatatatttccctgtttttctaaaaaagaaaaagatcatcattttcccattgtaaaatgccatatttttttcataggtcacttacatatatcaatgggtctgtttctgagctctactctattttatcagcctcactgtctatccccacacatctcatgctttgctctaaatcttgatatttagtggaacattctttcccattttgttctacaagaatatttttgttattgtctttgggctttctatatacattttgaaatgaggttgacaagttacctaggaaaactgtcttcataatcaacctctggattacaaaatttgtgaaagattgactggtattcttaactatgttgctccttttacgctatgtggatacgctgctttaatgcctttgtatcatgctattgcttcccgtatggctttcattttctcctccttgtataaatcctggttgctgtctctttatgaggagttgtggcccgttgtcaggcaacgtggcgtggtgtgcactgtgtttgctgacgcaacccccactggttggggcattgccaccacctgtcagctcctttccgggactttcgctttccccctccctattgccacggcggaactcatcgccgcctgccttgcccgctgctggacaggggctcggctgttgggcactgacaattccgtggtgttgtcggggaaatcatcgtcctttccttggctgctcgcctgtgttgccacctggattctgcgcgggacgtccttctgctacgtcccttcggccctcaatccagcggaccttccttcccgcggcctgctgccggctctgcggcctcttccgcctcttcgccttcgccctcagacgagtcggatctccctttgggccgcctccccgcatctggctaataaaggaaatttattttcattgcaatagtgtgttggaattttttgtgtctctcactcggaaggacatatgggagggcaaatcatttaaaacatcagaatgagtatttggtttagagtttggcaacatatgcccatatgctggctgccatgaacaaaggttggctataaagaggtcatcagtatatgaaacagccccctgctgtccattccttattccatagaaaagccttgacttgaggttagattttttttatattttgttttgtgttatttttttctttaacatccctaaaattttccttacatgttttactagccagatttttcctcctctcctgactactcccagtcatagctgtccctcttctcttatggagatcgaagacagtcag

SEQ ID NO: 55 - DNA, 643 bp, Artificial Sequence
  Made in Lab - Polynucleotide cassette 15 full 5'
ctctggagacgacttacggtaaatggcccgcctggctgaccgcccaacgacccccgcccattgacgtcaataatgacgtatgttcccatagtaacgccaatagggactttccattgacgtcaatgggtggagtatttacggtaaactgcccacttggcagtacatcaagtgtatcatatgccaagtccgccccctattgacgtcaatgacggtaaatggcccgcctggcattatgcccagtacatgaccttacgggactttcctacttggcagtacatctacgtattagtcatcgctattaccatgctgatgcggttttggcagtacaccaatgggcgtggatagcggtttgactcacggggatttccaagtctccaccccattgacgtcaatgggagtttgttttggcaccaaaatcaacgggactttccaaaatgtcgtaataaccccgccccgttgacgcaaatgggcggtaggcgtgtacggtgggaggtctatataagcagagctcgtttagtgaaccgtcagatcgcctggagaggccatccacgctgttttgacctccatagtggacaccgggaccgatccagcctccgcgtctcaggggagatctacacccaagctgtctagagccgccaccatg

SEQ ID NO: 56 - DNA, 1953 bp, Artificial Sequence
  Made in Lab - Polynucleotide cassette 15 full 3'
ctgttctcatcacatcatatcaaggttatataccatcaatattgccacagatgttacttagccttttaatatttctctaatttagtgtatatgcaatgatagttctctgatttctgagattgagtttctcatgtgtaatgattatttagagtttctctttcatctgttcaaatttttgtctagttttattttttactgatttgtaagacttctttttataatctgcatattacaattctctttactggggtgttgcaaatattttctgtcattctatggcctgacttttcttaatggttttttaattttaaaaataagtcttaatattcatgcaatctaattaacaatcttttctttgtggttaggactttgagtcataagaaatttttctctacactgaagtcatgatggcatgcttctatattattttctaaaagatttaaagttttgccttctccatttagacttataattcactggaatttttttgtgtgtatggtatgacatatgggttcccttttattttttacatataaatatatttccctgtttttctaaaaaagaaaaagatcatcattttcccattgtaaaatgccatatttttttcataggtcacttacatatatcaatgggtctgtttctgagctctactctattttatcagcctcactgtctatccccacacatctcatgctttgctctaaatcttgatatttagtggaacattctttcccattttgttctacaagaatatttttgttattgtctttgggctttctatatacattttgaaatgaggttgacaagttacctaggaaaactgtcttcataacaggcctattgattggaaagtttgtcaacgaattgtgggtcttttggggtttgctgccccttttacgcaatgtggatatcctgctttaatgcctttatatgcatgtatacaagcaaaacaggcttttactttctcgccaacttacaaggcctttctcagtaaacagtatatgaccctttaccccgttgctcggcaacggcctggtctgtgccaagtgtttgctgacgcaacccccactggttggggcttggccataggccatcagcgcatgcgtggaacctttgtgtctcctctgccgatccatactgcggaactcctagccgcttgttttgctcgcagcaggtctggagcaaacctcatcgggaccgacaattctgtcgtactctcccgcaagtatacatcgtttccatggctgctaggctgtgctgccaactggatcctgcgcgggacgtcctttgtttacgtcccgtcggcgctgaatcccgcggacgacccctcccggggccgcttggggctctaccgcccgcttctccgtctgccgtaccgtccgaccacggggcgcacctctctttacgcggactccccgtctgtgccttctcatctgccggaccgtgtgcacttcgcttcacctctgcacgtcgcatggaggccaccgtgaacgcccaccggaacctgcccaaggtcttgcataagaggactcttggactttcagcaatgtcatctggctaataaaggaaatttattttcattgcaatagtgtgttggaattttttgtgtctctcactcggaaggacatatgggagggcaaatcatttaaaacatcagaatgagtatttggtttagagtttggcaacatatgcccatatgctggctgccatgaacaaaggttggctataaagaggtcatcagtatatgaaacagccccctgctgtccattccttattccatagaaaagccttgacttgaggttagattttttttatattttgttttgtgttatttttttctttaacatccctaaaattttccttacatgttttactagccagatttttcctcctctcctgactactcccagtcatagctgtccctcttctcttatggagatcgaagacagtcag

SEQ ID NO: 57 - DNA, 673 bp, Artificial Sequence
  Made in Lab - Polynucleotide cassette 16 full 5'
ctctggagacgacttacggtaaatggcccgcctggctgaccgcccaacgacccccgcccattgacgtcaataatgacgtatgttcccatagtaacgccaatagggactttccattgacgtcaatgggtggagtatttacggtaaactgcccacttggcagtacatcaagtgtatcatatgccaagtccgccccctattgacgtcaatgacggtaaatggcccgcctggcattatgcccagtacatgaccttacgggactttcctacttggcagtacatctacgtattagtcatcgctattaccatgctgatgcggttttggcagtacaccaatgggcgtggatagcggtttgactcacggggatttccaagtctccaccccattgacgtcaatgggagtttgttttggcaccaaaatcaacgggactttccaaaatgtcgtaataaccccgccccgttgacgcaaatgggcggtaggcgtgtacggtgggaggtctatataagcagagctcgtttagtgaaccgtcagatcgcctggagaggccatccacgctgttttgacctccatagtggacaccgggaccgatccagcctccgcgtctcaggggagatctagcttgcttgttctttttgcagaagctcagaataaacgctcaactttggccgccaccatg

SEQ ID NO: 58 - DNA, 1690 bp, Artificial Sequence
  Made in Lab - Polynucleotide cassette 16 full 3'
ctgttctcatcacatcatatcaaggttatataccatcaatattgccacagatgttacttagccttttaatatttctctaatttagtgtatatgcaatgatagttctctgatttctgagattgagtttctcatgtgtaatgattatttagagtttctctttcatctgttcaaatttttgtctagttttattttttactgatttgtaagacttctttttataatctgcatattacaattctctttactggggtgttgcaaatattttctgtcattctatggcctgacttttcttaatggttttttaattttaaaaataagtcttaatattcatgcaatctaattaacaatcttttctttgtggttaggactttgagtcataagaaatttttctctacactgaagtcatgatggcatgcttctatattattttctaaaagatttaaagttttgccttctccatttagacttataattcactggaatttttttgtgtgtatggtatgacatatgggttcccttttattttttacatataaatatatttccctgtttttctaaaaaagaaaaagatcatcattttcccattgtaaaatgccatatttttttcataggtcacttacatatatcaatgggtctgtttctgagctctactctattttatcagcctcactgtctatccccacacatctcatgctttgctctaaatcttgatatttagtggaacattctttcccattttgttctacaagaatatttttgttattgtctttgggctttctatatacattttgaaatgaggttgacaagttacctaggaaaactgtcttcatataatcaacctctggattacaaaatttgtgaaagattgactggtattcttaactatgttgctccttttacgctatgtggatacgctgctttaatgcctttgtatcatgctattgcttcccgtatggctttcattttctcctccttgtataaatcctggttgctgtctctttatgaggagttgtggcccgttgtcaggcaacgtggcgtggtgtgcactgtgtttgctgacgcaacccccactggttggggcattgccaccacctgtcagctcctttccgggactttcgctttccccctccctattgccacggcggaactcatcgccgcctgccttgcccgctgctggacaggggctcggctgttgggcactgacaattccgtggtgttgtcggggaaatcatcgtcctttccttggctgctcgcctgtgttgccacctggattctgcgcgggacgtccttctgctacgtcccttcggccctcaatccagcggaccttccttcccgcggcctgctgccggctctgcggcctcttccgcctcttcgccttcgccctcagacgagtcggatctccctttgggccgcctccccgcatcatcttgccagccatctgttgtttgcccctcccccgtgccttccttgaccctggaaggtgccactcccactgtcctttcctaataaaatgaggaaattgcatcgcattgtctgagtaggtgtcattctattctggggggtggggtggggcaggacagcaagggggaggattgggaatacaatagcaggcatgctggggatgcggtgggctctatgggtacccaggtgctgaagaattgacccggttcctcctggggaagacagtcag

SEQ ID NO: 59 - DNA, 1126 bp, Artificial Sequence
  Made in Lab - Polynucleotide cassette 17 full 5'
ctctggagacgacttacggtaaatggcccgcctggctgaccgcccaacgacccccgcccattgacgtcaataatgacgtatgttcccatagtaacgccaatagggactttccattgacgtcaatgggtggagtatttacggtaaactgcccacttggcagtacatcaagtgtatcatatgccaagtccgccccctattgacgtcaatgacggtaaatggcccgcctggcattatgcccagtacatgaccttacgggactttcctacttggcagtacatctacgtattagtcatcgctattaccaatgacgtcgaggagaagttccccaactttcccgcctctcagcctttgaaagaaagaaaggggagggggcaggccgcgtgcagccgcgagcggtgctgggctccggctccaattccccatctcagtcgttcccaaagtcctcctgtttcatccaagcgtgtaagggtccccgtccttgactccctagtgtcctgctgcccacagtccagtcctgggaaccagcaccgatcacctcccatcgggccaatctcagtcccttcccccctacgtcggggcccacacgctcggtgcgtgcccagttgaaccaggcggctgcggaaaaaaaaaagcggggagaaagtagggcccggctactagcggttttacgggcgcacgtagctcaggcctcaagaccttgggctgggactggctgagcctggcgggaggcggggtccgagtcaccgcctgccgccgcgcccccggtttctataaattgagcccgcagcctcccgcttcgctctctgctcctcctgttcgacagtcagccgcatcttcttttgcgtcgccagcctggcagaactcggtaagtctgttgacatgtatgtgatgtatactaacctgcatgggacgtggatttacttgtgtatgtcagatagagtaaagattaactcttgcatgtgagcggggcatcgagatagcgataaatgagtcaggaggacggatacttatatgtgttgttatcctcctctacagtcaaacagattaagcgtctcaggggagatctagcttgcttgttctttttgcagaagctcagaataaacgctcaactttggccgccaccatg

SEQ ID NO: 60 - DNA, 1126 bp, Artificial Sequence
  Made in Lab - Polynucleotide cassette 17 full 3'
ggttcccttttattttttacatataaatatatttccctgtttttctaaaaaagaaaaagatcatcattttcccattgtaaaatgccatatttttttcataggtcacttacatatatcaatgggtctgtttctgagctctactctattttatcagcctcactgtctatccccacacatctcatgctttgctctaaatcttgatatttagtggaacattctttcccattttgttctacaagaatatttttgttattgtctttgggctttctatatacattttgaaatgaggttgacaagttacctaggaaaactgtcttcataatcaacctctggattacaaaatttgtgaaagattgactggtattcttaactatgttgctccttttacgctatgtggatacgctgctttaatgcctttgtatcatgctattgcttcccgtatggctttcattttctcctccttgtataaatcctggttgctgtctctttatgaggagttgtggcccgttgtcaggcaacgtggcgtggtgtgcactgtgtttgctgacgcaacccccactggttggggcattgccaccacctgtcagctcctttccgggactttcgctttccccctccctattgccacggcggaactcatcgccgcctgccttgcccgctgctggacaggggctcggctgttgggcactgacaattccgtggtgttgtcggggaaatcatcgtcctttccttggctgctcgcctgtgttgccacctggattctgcgcgggacgtccttctgctacgtcccttcggccctcaatccagcggaccttccttcccgcggcctgctgccggctctgcggcctcttccgcctcttcgccttcgccctcagacgagtcggatctccctttgggccgcctccccgcatcctgcccgggtggcatccctgtgacccctccccagtgcctctcctggccctggaagttgccactccagtgcccaccagccttgtcctaataaaattaagttgcatcattttgtctgactaggtgtccttctataatattatggggtggaggggggtggtatggagcaaggggcccaagttgggaagaaacctgtagggcctgcgaagacagtcag

SEQ ID NO: 61 - DNA, 820 bp, Artificial Sequence; identical to SEQ ID NO: 51
  Made in Lab - Polynucleotide cassette 18 full 5'

SEQ ID NO: 62 - DNA, 1091 bp, Artificial Sequence
  Made in Lab - Polynucleotide cassette 18 full 3'
ctgttctcatcacatcatatcaaggttatataccatcaatattgccacagatgttacttagccttttaatatttctctaatttagtgtatatgcaatgatagttctctgatttctgagattgagtttctcatgtgtaatgattatttagagtttctctttcatctgttcaaatttttgtctagttttattttttactgatttgtaagacttctttttataatctgcatattacaattctctttactggggtgttgcaaatattttctgtcattctatggcctgacttttcttaatggttttttaattttaaaaataagtcttaatattcatgcaatctaattaacaatcttttctttgtggttaggactttgagtcataagaaatttttctctacactgaagtcatgatggcatgcttctatattattttctaaaagatttaaagttttgccttctccatttagacttataattcactggaatttttttgtgtgtatggtatgacatatgggttcccttttattttttacatataaatatatttccctgtttttctaaaaaagaaaaagatcatcattttcccattgtaaaatgccatatttttttcataggtcacttacatatatcaatgggtctgtttctgagctctactctattttatcagcctcactgtctatccccacacatctcatgctttgctctaaatcttgatatttagtggaacattctttcccattttgttctacaagaatatttttgttattgtctttgggctttctatatacattttgaaatgaggttgacaagttacctaggaaaactgtcttcttgccagccatctgttgtttgcccctcccccgtgccttccttgaccctggaaggtgccactcccactgtcctttcctaataaaatgaggaaattgcatcgcattgtctgagtaggtgtcattctattctggggggtggggtggggcaggacagcaagggggaggattgggaatacaatagcaggcatgctggggatgcggtgggctctatgggtacccaggtgctgaagaattgacccggttcctcctggggaagacagtcag

SEQ ID NO: 63 - skipped

SEQ ID NO: 64 - DNA, 151 bp, Artificial Sequence
  Made in Lab - Cassette 7 Enhancer Promoter Junction
gcccgcctggcattatgcccagtacatgaccttatgggactttcctacttggcagtacatctacgtattagtcatcgctattaccatggtcgaggtgagccccacgttctgcttcactctccccatctcccccccctccccacccccaatt

SEQ ID NO: 65 - DNA, 151 bp, Artificial Sequence
  Made in Lab - Cassette 7 Promoter Intro Junction
tccgaaagtttccttttatggcgaggcggcggcggcggcggccctataaaaagcgaagcgcgcggcgggcgggagtcgctgcgcgctgccttcgccccgtgccccgctccgccgccgcctcgcgccgcccgccccggctctgactgaccgc

SEQ ID NO: 66 - DNA, 86 bp, Artificial Sequence
  Made in Lab - Cassette 7 Intron 5' UTR Junction
agctcctgggcaacgtgctggttattgtgctgtctcatcattttggcaaagaattcggcttgatcgaagccgtctcaggggagatc

SEQ ID NO: 67 - DNA, 41 bp, Artificial Sequence
  Made in Lab - Cassette 7 UTR Kozak junction
tttttgcagaagctcagaataaacgctcaactttggccgcc

SEQ ID NO: 68 - DNA, 90 bp, Artificial Sequence
  Made in Lab - Cassette 7 Enhancer RNA Export  Junction
ccctgtttttctaaaaaagacctaggaaaactgtcttcataacaggcctattgattggaaagtttgtcaacgaattgtgggtcttttggg

SEQ ID NO: 69 - DNA, 90 bp, Artificial Sequence; identical to SEQ ID NO: 68
  Made in Lab - Cassette 7 RNA Export PolyA Junction

SEQ ID NO: 70 - DNA, 100 bp, Artificial Sequence
  Made in Lab - Cassette 10 Enhancer Promoter Junction
cgggactttcctacttggcagtacatctacgtattagtcatcgctattaccagcacatcgcccacagtccccgagaagttggggggaggggtcggcaatt

SEQ ID NO: 71 - DNA, 120 bp, Artificial Sequence
  Made in Lab - Cassette 10 Promoter Intron Junction
gggtgggggagaaccgtatataagtgcagtagtcgccgtgaacgttctttttcgcaacgggtttgccgccagaacacaggtaagtgccgtgtgtggttcccgcgggcctggcctctttac

SEQ ID NO: 72 - DNA, 55 bp, Artificial Sequence
  Made in Lab - Cassette 10 Intron UTR
gacagtggttcaaagtttttttcttccatttcaggtgtcctgaacacgtctcagg

SEQ ID NO: 73 - DNA, 15 bp, Artificial Sequence
  Made in Lab - Cassette 10 UTR Kozak junction
agctgtctagagccg

SEQ ID NO: 74 - DNA, 146 bp, Artificial Sequence
  Made in Lab - Cassette 10 Enhancer RNA Export  Junction
gtctttgggctttctatatacattttgaaatgaggttgacaagttacctaggaaaactgtcttcatataatcaacctctggattacaaaatttgtgaaagattgactggtattcttaactatgttgctccttttacgctatgtgga

SEQ ID NO: 75 - DNA, 98 bp, Artificial Sequence
  Made in Lab - Cassette 10 RNA Export PolyA Junction
cttcgccctcagacgagtcggatctccctttgggccgcctccccgcatcatcttgccagccatctgttgtttgcccctcccccgtgccttccttgacc

SEQ ID NO: 76 - DNA, 68 bp, Artificial Sequence
  Made in Lab - Cassette 11 TPL Enhancer junction
aggcggtcttgagacggcggatggtcgaggtgaggtgtggcaggcttgagatccagctgttggggtga

SEQ ID NO: 77 - DNA, 129 bp, Artificial Sequence
  Made in Lab - Cassette 11 Promoter TPL  Junction
cgctgttttgacctccatagtggacaccgggaccgatccagcctccgcgtctcaggggagatctcgtttagtgaaccgtcagatcctcactctcttccgcatcgctgtctgcgagggccagctgttggg

SEQ ID NO: 78 - DNA, 36 bp, Artificial Sequence
  Made in Lab - Cassette 11 Promoter Intron Junction
ttgatattcacctggcccgatctggccatacacttg

SEQ ID NO: 79 - DNA, 22 bp, Artificial Sequence
  Made in Lab - Cassette 11 UTR Kozak junction
cccaggtccaagtttaaacgcc

SEQ ID NO: 80 - DNA, 77 bp, Artificial Sequence
  Made in Lab - Cassette 11 Enhancer PolyA Junction
tctttgggctttctatatacattttgaaatgaggttgacaagttacctaggaaaactgtcttcctgcccgggtggca

SEQ ID NO: 81 - DNA, 149 bp, Artificial Sequence
  Made in Lab - Cassette 12 Promoter TPL Junction
tcagatcgcctggagaggccatccacgctgttttgacctccatagtggacaccgggaccgatccagcctccgcgtctcaggggagatctcgtttagtgaaccgtcagatcctcactctcttccgcatcgctgtctgcgagggccagctg

SEQ ID NO: 82 - DNA, 95 bp, Artificial Sequence
  Made in Lab - Cassette 12 TPL Enhancer Junction
gatgtaattaaagtaggcggtcttgagacggcggatggtcgaggtgaggtgtggcaggcttgagatccagctgttggggtgagtactccctctca

SEQ ID NO: 83 - DNA, 41 bp, Artificial Sequence
  Made in Lab - Cassette 12 Enhancer Intro Junction
gatttgatattcacctggcccgatctggccatacacttgag

SEQ ID NO: 84 - DNA, 29 bp, Artificial Sequence
  Made in Lab - Cassette 12 UTR Kozak junction
tgtccactcccaggtccaagtttaaacgc

SEQ ID NO: 85 - DNA, 76 bp, Artificial Sequence
  Made in Lab - Cassette 12 Enhancer RNA Export  Junction
tgtttttctaaaaaagacctaggaaaactgtcttcataacaggcctattgattggaaagtttgtcaacgaattgtg

SEQ ID NO: 86 - DNA, 110 bp, Artificial Sequence
  Made in Lab - Cassette 12 RNA Export PolyA Junction
aaggtcttgcataagaggactcttggactttcagcaatgtcatcttgccagccatctgttgtttgcccctcccccgtgccttccttgaccctggaaggtgccactcccac

SEQ ID NO: 87 - DNA, 110 bp, Artificial Sequence
  Made in Lab - Cassette 13 Promoter Enhancer Junction
gcggccctataaaaagcgaagcgcgcggcgggcggcgtctcaggggagatctggtgaggtgtggcaggcttgagatccagctgttggggtgagtactccctctcaaaagc

SEQ ID NO: 88 - DNA, 44 bp, Artificial Sequence
  Made in Lab - Cassette 13 Enhancer Intron Junction
ggaggatttgatattcacctggcccgatctggccatacacttga

SEQ ID NO: 89 - DNA, 49 bp, Artificial Sequence
  Made in Lab - Cassette 13 Intron Kozak Junction
cctttctctccacaggtgtccactcccaggtccaagtttaaacgccgcc

SEQ ID NO: 90 - DNA, 129 bp, Artificial Sequence
  Made in Lab - Cassette 13 Enhancer RNA Export  Junction
attgtctttgggctttctatatacattttgaaatgaggttgacaagttacctaggaaaactgtcttcataacaggcctattgattggaaagtttgtcaacgaattgtgggtcttttggggtttgctgcc

SEQ ID NO: 91 - DNA, 110 bp, Artificial Sequence
  Made in Lab - Cassette 13 RNA Export PolyA Junction
cctgcccaaggtcttgcataagaggactcttggactttcagcaatgtcatctggctaataaaggaaatttattttcattgcaatagtgtgttggaattttttgtgtctct

SEQ ID NO: 92 - DNA, 94 bp, Artificial Sequence
  Made in Lab - Cassette 14 Promoter Intron Junction
cggtgcattggaacgcggattccccgtgccaagagtgaccctggcagaactcggtaagtctgttgacatgtatgtgatgtatactaacctgcat

SEQ ID NO: 93 - DNA, 112 bp, Artificial Sequence
  Made in Lab - Cassette 14 Intron Kozak junction
acttatatgtgttgttatcctcctctacagtcaaacagattaagcgtctcaggggagatctagcttgcttgttctttttgcagaagctcagaataaacgctcaactttggcc

SEQ ID NO: 94 - DNA, 99 bp, Artificial Sequence
  Made in Lab - Cassette 14 Enhancer RNA Export  Junction
gctttctatatacattttgaaatgaggttgacaagttacctaggaaaactgtcttcataatcaacctctggattacaaaatttgtgaaagattgactgg

SEQ ID NO: 95 - DNA, 100 bp, Artificial Sequence
  Made in Lab - Cassette 14 RNA Export PolyA Junction
cttcgccttcgccctcagacgagtcggatctccctttgggccgcctccccgcatctggctaataaaggaaatttattttcattgcaatagtgtgttggaa

SEQ ID NO: 96 - DNA, 280 bp, Gallus gallus
tggtcgaggtgagccccacgttctgcttcactctccccatctcccccccctccccacccccaattttgtatttatttattttttaattattttgtgcagcgatgggggcggggggggggggggcgcgcgccaggcggggcggggcggggcgaggggcggggcggggcgaggcggagaggtgcggcggcagccaatcagagcggcgcgctccgaaagtttccttttatggcgaggcggcggcggcggcggccctataaaaagcgaagcgcgcggcgggcgg

SEQ ID NO: 97 - DNA, 973 bp, Gallus gallus
ggagtcgctgcgcgctgccttcgccccgtgccccgctccgccgccgcctcgcgccgcccgccccggctctgactgaccgcgttactcccacaggtgagcgggcgggacggcccttctcctccgggctgtaattagcgcttggtttaatgacggcttgtttcttttctgtggctgcgtgaaagccttgaggggctccgggagggccctttgtgcgggggggagcggctcggggggtgcgtgcgtgtgtgtgtgcgtggggagcgccgcgtgcggctccgcgctgcccggcggctgtgagcgctgcgggcgcggcgcggggctttgtgcgctccgcagtgtgcgcgaggggagcgcggccgggggcggtgccccgcggtgcggggggggctgcgaggggaacaaaggctgcgtgcggggtgtgtgcgtgggggggtgagcagggggtgtgggcgcgtcggtcgggctgcaaccccccctgcacccccctccccgagttgctgagcacggcccggcttcgggtgcggggctccgtacggggcgtggcgcggggctcgccgtgccgggcggggggtggcggcaggtgggggtgccgggcggggcggggccgcctcgggccggggagggctcgggggaggggcgcggcggcccccggagcgccggcggctgtcgaggcgcggcgagccgcagccattgccttttatggtaatcgtgcgagagggcgcagggacttcctttgtcccaaatctgtgcggagccgaaatctgggaggcgccgccgcaccccctctagcgggcgcggggcgaagcggtgcggcgccggcaggaaggaaatgggcggggagggccttcgtgcgtcgccgcgccgccgtccccttctccctctccagcctcggggctgtccgcggggggacggctgccttcgggggggacggggcagggcggggttcggcttctggcgtgtgaccggcggctct